European Patent Specification EP 4 301 870 B1, published January 15, 2025. Title: MULTIPLEX CAPTURE OF GENE AND PROTEIN EXPRESSION IN A BIOLOGICAL SAMPLE. Applicant: 10x Genomics, Inc. The sequence listing filed with the application follows.

SEQUENCE LISTING (11 sequences)

SEQ ID NO: 1 - DNA, 22 bp, Artificial
  Capture Domain 22mer
ttgctaggaccggccttaaagc

SEQ ID NO: 2 - DNA, 21 bp, Artificial
  Capture Domain 21mer
ttgctaggaccggccttaaag

SEQ ID NO: 3 - DNA, 20 bp, Artificial
  Capture Domain 20mer
ttgctaggaccggccttaaa

SEQ ID NO: 4 - DNA, 19 bp, Artificial
  Capture Domain 19mer
ttgctaggaccggccttaa

SEQ ID NO: 5 - DNA, 18 bp, Artificial
  Capture Domain 18mer
ttgctaggaccggcctta

SEQ ID NO: 6 - DNA, 17 bp, Artificial
  Capture Domain 17mer
ttgctaggaccggcctt

SEQ ID NO: 7 - DNA, 16 bp, Artificial
  Capture Domain 16mer
ttgctaggaccggcct

SEQ ID NO: 8 - DNA, 15 bp, Artificial
  Capture Domain 15mer
ttgctaggaccggcc

SEQ ID NO: 9 - DNA, 14 bp, Artificial
  Capture Domain 14mer
ttgctaggaccggc

SEQ ID NO: 10 - DNA, 13 bp, Artificial
  Capture Domain 13mer
ttgctaggaccgg

SEQ ID NO: 11 - DNA, 12 bp, Artificial
  Capture Domain 12mer
ttgctaggaccg